European Patent Application EP 4 417 626 A1, published August 21, 2024. Title: 新型抗体-细胞因子融合蛋白及其制备方法和用途. Applicant: 徕特康（苏州）生物制药有限公司. The sequence listing filed with the application follows.

SEQUENCE LISTING (237 sequences)

SEQ ID NO: 1 - protein, 133 aa, Homo sapiens [sequence omitted]

SEQ ID NO: 2 - protein, 133 aa, synthetic construct
  REGION 1..133: note = hIL2-DM
APTSSSTKKTQLQLEHLLLDLQMILNGINNYKNPKLTRMLTFKFYMPKKATELKHLQCLEEELGPLEEVLNLAQSKNFHLRPRDLISNIRVIVLELKGSETTFMCEYADETATIVEFLNRWITFCQSIISTLT

SEQ ID NO: 3 - protein, 133 aa, synthetic construct
  REGION 1..133: note = hIL2-TM
APTSSSTKKTQLQLEHLLLDLQMILNGINNYKNPKLTRMLTFKFYMPKKATELKHLQCLEEELGPLEEVLNLAQSKNFHLRPRDLISNIRVIVLELKGSETTFECEYADETATIVEFLNRWITFCQSIISTLT

SEQ ID NO: 4 - protein, 149 aa, Mus musculus
APTSSSTSSSTAEAQQQQQQQQQQQQHLEQLLMDLQELLSRMENYRNLKLPRMLTFKFYLPKQATELKDLQCLEDELGPLRHVLDLTQSKSFQLEDAENFISNIRVTVVKLKGSDNTFECQFDDESATVVDFLRRWIAFCQSIISTSPQ

SEQ ID NO: 5 - protein, 123 aa, synthetic construct
  REGION 1..123: note = S4B6 - VH
EVQLQESGAELVRPGTSVKLSCKVSGDTITAYYLHFVRQRPGQGLEWIGRIDPEDDSTKYAENFKNKATFTADASSNTAYLRLSSLTSEDTATYFCTTVTFYYSRELRWFAYWGQGTLVTVSS

SEQ ID NO: 6 - protein, 107 aa, synthetic construct
  REGION 1..107: note = S4B6 - VL
DIQVTQSPASLSASLEEIVTITCQASQDIGNYLSWYQQKLGKSPQLLIHSATSLADGVPSRFSGSRSGTQYSLKINRLQVEDTGIYYCLQHYSTPYTFGAGTKLELK

SEQ ID NO: 7 - protein, 5 aa, synthetic construct
  REGION 1..5: note = HCDR1 of S4B6, Humanized Antibodies, hS4B6-H6K3-hu01, hS4B6-H6K3-hu02 and hS4B6-H6K3-hu05 to hS4B6-H6K3-hu12
AYYLH

SEQ ID NO: 8 - protein, 17 aa, synthetic construct
  REGION 1..17: note = HCDR2 of S4B6, Humanized Antibodies, hS4B6-H6K3-hu01 to hS4B6-H6K3-hu05 and hS4B6-H6K3-hu08 to hS4B6-H6K3-hu12
RIDPEDDSTKYAENFKN

SEQ ID NO: 9 - protein, 14 aa, synthetic construct
  REGION 1..14: note = HCDR3 of S4B6, Humanized Antibodies, hS4B6-H6K3-hu01 to hS4B6-H6K3-hu12, hS4B6-H6K3(H), K1G1, K1G3, K2G1, K2G3, K3G1, K3G3, K4G1, K4G3, and H6K3(H)-Cy01 to H6K3(H)-Cy06
VTFYYSRELRWFAY

SEQ ID NO: 10 - protein, 11 aa, synthetic construct
  REGION 1..11: note = LCDR1 of S4B6, Humanized Antibody, hS4B6-H6K3-hu01 to hS4B6-H6K3-hu12, hS4B6-H6K3(H), H6K3(H)-Cy03 to H6K3(H)-Cy08, H6K3(H)-Cy10, and H6K3(H)-Cy08-DE
QASQDIGNYLS

SEQ ID NO: 11 - protein, 7 aa, synthetic construct
  REGION 1..7: note = LCDR2 of S4B6, Humanized Antibodies, hS4B6-H6K3-hu01 to hS4B6-H6K3-hu08, hS4B6-H6K3-hu11 to hS4B6-H6K3-hu12
SATSLAD

SEQ ID NO: 12 - protein, 9 aa, synthetic construct
  REGION 1..9: note = LCDR3 of S4B6, Humanized Antibodies, hS4B6-H6K3-hu01 to hS4B6-H6K3-hu12, hS4B6-H6K3(H), Antibodies engineered by Affinity maturation, H6K3(H)-Cy01 to H6K3(H)-Cy08 and H6K3(H)-Cy10, Each Mutant of H6K3(H)-Cy08, and K2G11-Cy01 to K2G11-Cy08 and K2G11-Cy10 to K2G11-Cy12
LQHYSTPYT

SEQ ID NO: 13 - protein, 5 aa, synthetic construct
  REGION 1..5: note = HCDR1 of Deeply Humanized Antibody hS4B6-H6K3-hu03
DYYLH

SEQ ID NO: 14 - protein, 5 aa, synthetic construct
  REGION 1..5: note = HCDR1 of hS4B6-H6K3-hu04, hS4B6-H6K3(H), Antibodies engineered by Affinity maturation, H6K3(H)-Cy-01 to H6K3(H)-Cy-08 and H6K3(H)-Cy-10, Each Mutant of H6K3(H)-Cy-08, and K2G11-Cy01 to K2G11-Cy12
AYYMH

SEQ ID NO: 15 - protein, 17 aa, synthetic construct
  REGION 1..17: note = HCDR2 of H6K3-hu07, H6K3 (H), K1G1, K1G2, K1G4, K1G5, K1G7, K1G8, K1G9; K2G1, K2G2, K2G4, K2G5, K2G7, K2G8, K2G9; K3G1, K3G2, K3G4, K3G5, K3G7, K3G8, K3G9; K4G1, K4G2, K4G4, K4G5, K4G7, K4G8, K4G9; H6K3(H)-Cy-01 to H6K3(H)-Cy08 and H6K3(H)-Cy10, Each Mutant of H6K3(H)-Cy08
RIDPEDDSTKYAENFKG

SEQ ID NO: 16 - protein, 17 aa, synthetic construct
  REGION 1..17: note = HCDR2 of hS4B6-H6K3-hu06
RIDPEDDSTKYAENFKS

SEQ ID NO: 17 - protein, 7 aa, synthetic construct
  REGION 1..7: note = LCDR2 of hS4B6-H6K3-hu09, hS4B6-H6K3(H), K2G1 to K2G12, K4G1 to K4G12, H6K3(H)-Cy01, H6K3(H)-Cy02, H6K3(H)-Cy05 to H6K3(H)-Cy08 and H6K3(H)-Cy10, Each Mutant of H6K3(H)-Cy08, K2G11-Cy01, K2G11-Cy02, and K2G11-Cy05 to K2G11-Cy12
SATSLAS

SEQ ID NO: 18 - protein, 7 aa, synthetic construct
  REGION 1..7: note = LCDR2 of hS4B6-H6K3-hu10
SATSLAT

SEQ ID NO: 19 - protein, 17 aa, synthetic construct
  REGION 1..17: note = HCDR2 of K1G3, K1G6, K1G10, K1G11, K1G12, K2G3, K2G6, K2G10, K2G11, K2G12, K3G3, K3G6, K3G10, K3G11, K3G12, K4G3, K4G6, K4G10, K4G11, K4G12,and K2G11-Cy01 to K2G11-Cy12
RIDPDDDSTKYAENFKG

SEQ ID NO: 20 - protein, 14 aa, synthetic construct
  REGION 1..14: note = HCDR3 of K1G2, K1G6, K2G2, K2G6, K3G2, K3G6, K4G2, and K4G6
ITFYYSRELRWFAY

SEQ ID NO: 21 - protein, 14 aa, synthetic construct
  REGION 1..14: note = HCDR3 of K1G4, K2G4, K3G4, and K4G4
VTFLYSRELRWFAY

SEQ ID NO: 22 - protein, 14 aa, synthetic construct
  REGION 1..14: note = HCDR3 of K1G5, K2G5, K3G5, and K4G5
VTFYYTRELRWFAY

SEQ ID NO: 23 - protein, 14 aa, synthetic construct
  REGION 1..14: note = HCDR3 of K1G7, K1G10, K2G7, K2G10, K3G7, K3G10, K3G7, K3G10, K4G7, and K4G10
ITFYYTRELRWFAY

SEQ ID NO: 24 - protein, 14 aa, synthetic construct
  REGION 1..14: note = HCDR3 of K1G8, K1G11, K2G8, K2G11, K3G8, K3G11, K4G8, K4G11, K2G11-Cy01 to K2G11-Cy06, K2G11-Cy09, K2G11-Cy11, and K2G11-Cy12
ITFLYSRELRWFAY

SEQ ID NO: 25 - protein, 14 aa, synthetic construct
  REGION 1..14: note = HCDR3 of K1G9, K1G12, K2G9, K2G12, K3G9, K3G12, K4G9, and K4G12
ITFLYTRELRWFAY

SEQ ID NO: 26 - protein, 11 aa, synthetic construct
  REGION 1..11: note = LCDR1 of K1G1 to K1G12, K2G2 to K2G12, and K2G11-Cy03 to K2G11-Cy10
QASQYISNYLS

SEQ ID NO: 27 - protein, 11 aa, synthetic construct
  REGION 1..11: note = LCDR1 of K3G1 to K3G12, and K4G1 to K4G12
QASQYIGNYLS

SEQ ID NO: 28 - protein, 7 aa, synthetic construct
  REGION 1..7: note = LCDR2 of K1G1 to K1G12, and K3G1 to K3G12
QATSLAS

SEQ ID NO: 29 - protein, 14 aa, synthetic construct
  REGION 1..14: note = HCDR3 of H6K3(H)-Cy07, H6K3(H)-Cy08, H6K3(H)-Cy10, and Each Mutant of H6K3(H)-Cy08
VTCYYSRELRWFAY

SEQ ID NO: 30 - protein, 11 aa, synthetic construct
  REGION 1..11: note = LCDR1 of H6K3(H)-Cy01
QASQDICNYLS

SEQ ID NO: 31 - protein, 11 aa, synthetic construct
  REGION 1..11: note = LCDR1 of H6K3(H)-Cy02
QASQDIGCYLS

SEQ ID NO: 32 - protein, 7 aa, synthetic construct
  REGION 1..7: note = LCDR2 of H6K3(H)-Cy03 and K2G11-Cy03
CATSLAS

SEQ ID NO: 33 - protein, 7 aa, synthetic construct
  REGION 1..7: note = LCDR2 of H6K3(H)-Cy04 and K2G11-Cy04
SACSLAS

SEQ ID NO: 34 - protein, 14 aa, synthetic construct
  REGION 1..14: note = HCDR3 of K2G11-Cy07, K2G11-Cy08, and K2G11-Cy10
ITCLYSRELRWFAY

SEQ ID NO: 35 - protein, 11 aa, synthetic construct
  REGION 1..11: note = LCDR1 of K2G11-Cy01 and K2G11-Cy11
QASQYICNYLS

SEQ ID NO: 36 - protein, 11 aa, synthetic construct
  REGION 1..11: note = LCDR1 of K2G11-Cy02
QASQYISCYLS

SEQ ID NO: 37 - protein, 11 aa, synthetic construct
  REGION 1..11: note = LCDR1 of K2G11-Cy12
QASQYISNCLS

SEQ ID NO: 38 - protein, 9 aa, synthetic construct
  REGION 1..9: note = LCDR3 of K2G11-Cy09
LQHCSTPYT

SEQ ID NO: 39 - protein, 11 aa, synthetic construct
  REGION 1..11: note = LCDR1 of H6K3(H)-Cy08-QD
QASDDIGNYLS

SEQ ID NO: 40 - protein, 11 aa, synthetic construct
  REGION 1..11: note = LCDR1 of H6K3(H)-Cy08-QE
QASEDIGNYLS

SEQ ID NO: 41 - protein, 11 aa, synthetic construct
  REGION 1..11: note = LCDR1 of H6K3(H)-Cy08-QS
QASSDIGNYLS

SEQ ID NO: 42 - protein, 11 aa, synthetic construct
  REGION 1..11: note = LCDR1 of H6K3(H)-Cy08-QG
QASGDIGNYLS

SEQ ID NO: 43 - protein, 11 aa, synthetic construct
  REGION 1..11: note = LCDR1 of H6K3(H)-Cy08-QK
QASKDIGNYLS

SEQ ID NO: 44 - protein, 11 aa, synthetic construct
  REGION 1..11: note = LCDR1 of H6K3(H)-Cy08-QR
QASRDIGNYLS

SEQ ID NO: 45 - protein, 123 aa, synthetic construct
  REGION 1..123: note = hS4B6-H1
QVQLQESGPGLVKPSETLSLTCTVSGDTITAYYLHWIRQPPGKGLEWIGRIDPEDDSTKYAENFKNRVTISVDTSKNQFSLKLSSVTAADTAVYYCTTVTFYYSRELRWFAYWGQGTTVTVSS

SEQ ID NO: 46 - protein, 107 aa, synthetic construct
  REGION 1..107: note = hS4B6-K1
DIVLTQSPGTLSLSPGERATLSCQASQDIGNYLSWYQQKPGQAPRLLIYSATSLADGIPDRFSGSRSGTDYTLTISRLEPEDFAVYYCLQHYSTPYTFGQGTKVEIK

SEQ ID NO: 47 - protein, 123 aa, synthetic construct
  REGION 1..123: note = hS4B6-H3
QVTLKESGPVLVKPTQTLTLTCTVSGDTITAYYLHWIRQPPGKALEWIGRIDPEDDSTKYAENFKNRLTFSADTSKNQVVLTMTNMDPVDTATYYCARVTFYYSRELRWFAYWGQGTLVTVSS

SEQ ID NO: 48 - protein, 107 aa, synthetic construct
  REGION 1..107: note = hS4B6-K3
DIVLTQSPATLSLSPGERATLSCQASQDIGNYLSWYQQKPGQAPRLLIYSATSLADGIPARFSGSRSGTDYTLTISSLEPEDFAVYYCLQHYSTPYTFGQGTKLEIK

SEQ ID NO: 49 - protein, 123 aa, synthetic construct
  REGION 1..123: note = hS4B6-H6
QVQLVQSGAEVKKPGATVKISCKVSGDTITAYYLHWVRQAPGQGLEWIGRIDPEDDSTKYAENFKNRVTITADTSTNTAYMELSSLRSEDTAVYYCTTVTFYYSRELRWFAYWGQGTLVTVSS

SEQ ID NO: 50 - protein, 107 aa, synthetic construct
  REGION 1..107: note = hS4B6-K7
DIQMTQSPSSLSASVGDRVTITCQASQDIGNYLSWYQQKPGKAPKLLIHSATSLADGVPSRFSGSGSGTDFTLTISSLQPEDFATYYCLQHYSTPYTFGGGTKVEIK

SEQ ID NO: 51 - protein, 123 aa, synthetic construct
  REGION 1..123: note = H6K3-hu01-VH
QVQLVQSGAEVKKPGATVKISCKVSGYTITAYYLHWVRQAPGQGLEWIGRIDPEDDSTKYAENFKNRVTITADTSTNTAYMELSSLRSEDTAVYYCTTVTFYYSRELRWFAYWGQGTLVTVSS

SEQ ID NO: 52 - protein, 123 aa, synthetic construct
  REGION 1..123: note = H6K3-hu02-VH
QVQLVQSGAEVKKPGATVKISCKVSGDTFTAYYLHWVRQAPGQGLEWIGRIDPEDDSTKYAENFKNRVTITADTSTNTAYMELSSLRSEDTAVYYCTTVTFYYSRELRWFAYWGQGTLVTVSS

SEQ ID NO: 53 - protein, 123 aa, synthetic construct
  REGION 1..123: note = H6K3-hu03-VH
QVQLVQSGAEVKKPGATVKISCKVSGDTITDYYLHWVRQAPGQGLEWIGRIDPEDDSTKYAENFKNRVTITADTSTNTAYMELSSLRSEDTAVYYCTTVTFYYSRELRWFAYWGQGTLVTVSS

SEQ ID NO: 54 - protein, 123 aa, synthetic construct
  REGION 1..123: note = H6K3-hu04-VH
QVQLVQSGAEVKKPGATVKISCKVSGDTITAYYMHWVRQAPGQGLEWIGRIDPEDDSTKYAENFKNRVTITADTSTNTAYMELSSLRSEDTAVYYCTTVTFYYSRELRWFAYWGQGTLVTVSS

SEQ ID NO: 55 - protein, 123 aa, synthetic construct
  REGION 1..123: note = H6K3-hu05-VH
QVQLVQSGAEVKKPGATVKISCKVSGDTITAYYLHWVRQAPGQGLEWMGRIDPEDDSTKYAENFKNRVTITADTSTNTAYMELSSLRSEDTAVYYCTTVTFYYSRELRWFAYWGQGTLVTVSS

SEQ ID NO: 56 - protein, 123 aa, synthetic construct
  REGION 1..123: note = H6K3-hu06-VH
QVQLVQSGAEVKKPGATVKISCKVSGDTITAYYLHWVRQAPGQGLEWIGRIDPEDDSTKYAENFKSRVTITADTSTNTAYMELSSLRSEDTAVYYCTTVTFYYSRELRWFAYWGQGTLVTVSS

SEQ ID NO: 57 - protein, 123 aa, synthetic construct
  REGION 1..123: note = H6K3-hu07-VH
QVQLVQSGAEVKKPGATVKISCKVSGDTITAYYLHWVRQAPGQGLEWIGRIDPEDDSTKYAENFKGRVTITADTSTNTAYMELSSLRSEDTAVYYCTTVTFYYSRELRWFAYWGQGTLVTVSS

SEQ ID NO: 58 - protein, 123 aa, synthetic construct
  REGION 1..123: note = H6K3-hu08-VH
QVQLVQSGAEVKKPGATVKISCKVSGDTITAYYLHWVRQAPGQGLEWIGRIDPEDDSTKYAENFKNRVTITADTSTDTAYMELSSLRSEDTAVYYCTTVTFYYSRELRWFAYWGQGTLVTVSS

SEQ ID NO: 59 - protein, 107 aa, synthetic construct
  REGION 1..107: note = H6K3-hu09-VL
DIVLTQSPATLSLSPGERATLSCQASQDIGNYLSWYQQKPGQAPRLLIYSATSLASGIPARFSGSRSGTDYTLTISSLEPEDFAVYYCLQHYSTPYTFGQGTKLEIK

SEQ ID NO: 60 - protein, 107 aa, synthetic construct
  REGION 1..107: note = H6K3-hu10-VL
DIVLTQSPATLSLSPGERATLSCQASQDIGNYLSWYQQKPGQAPRLLIYSATSLATGIPARFSGSRSGTDYTLTISSLEPEDFAVYYCLQHYSTPYTFGQGTKLEIK

SEQ ID NO: 61 - protein, 107 aa, synthetic construct
  REGION 1..107: note = H6K3-hu11-VL
DIVLTQSPATLSLSPGERATLSCQASQDIGNYLSWYQQKPGQAPRLLIYSATSLADGIPARFSGSGSGTDYTLTISSLEPEDFAVYYCLQHYSTPYTFGQGTKLEIK

SEQ ID NO: 62 - protein, 107 aa, synthetic construct
  REGION 1..107: note = H6K3-hu12-VL
DIVLTQSPATLSLSPGERATLSCQASQDIGNYLSWYQQKPGQAPRLLIYSATSLADGIPARFSGSRSGTDFTLTISSLEPEDFAVYYCLQHYSTPYTFGQGTKLEIK

SEQ ID NO: 63 - protein, 123 aa, synthetic construct
  REGION 1..123: note = VH of hS4B6-H6K3(H), K1G1, K2G1, K3G1, K4G1, and H6K3(H)-Cy01 to H6K3(H)-Cy06
QVQLVQSGAEVKKPGATVKISCKVSGDTITAYYMHWVRQAPGQGLEWIGRIDPEDDSTKYAENFKGRVTITADTSTDTAYMELSSLRSEDTAVYYCTTVTFYYSRELRWFAYWGQGTLVTVSS

SEQ ID NO: 64 - protein, 107 aa, synthetic construct
  REGION 1..107: note = VL of hS4B6-H6K3(H), H6K3(H)-Cy07, H6K3(H)-Cy08, and H6K3(H)-Cy10
DIVLTQSPATLSLSPGERATLSCQASQDIGNYLSWYQQKPGQAPRLLIYSATSLASGIPARFSGSRSGTDFTLTISSLEPEDFAVYYCLQHYSTPYTFGQGTKLEIK

SEQ ID NO: 65 - protein, 123 aa, synthetic construct
  REGION 1..123: note = VH of K1G2, K2G2, K3G2, K4G2
QVQLVQSGAEVKKPGATVKISCKVSGDTITAYYMHWVRQAPGQGLEWIGRIDPEDDSTKYAENFKGRVTITADTSTDTAYMELSSLRSEDTAVYYCTTITFYYSRELRWFAYWGQGTLVTVSS

SEQ ID NO: 66 - protein, 123 aa, synthetic construct
  REGION 1..123: note = VH of K1G3, K2G3, K3G3, K4G3
QVQLVQSGAEVKKPGATVKISCKVSGDTITAYYMHWVRQAPGQGLEWIGRIDPDDDSTKYAENFKGRVTITADTSTDTAYMELSSLRSEDTAVYYCTTVTFYYSRELRWFAYWGQGTLVTVSS

SEQ ID NO: 67 - protein, 123 aa, synthetic construct
  REGION 1..123: note = VH of K1G4, K2G4, K3G4, K4G4
QVQLVQSGAEVKKPGATVKISCKVSGDTITAYYMHWVRQAPGQGLEWIGRIDPEDDSTKYAENFKGRVTITADTSTDTAYMELSSLRSEDTAVYYCTTVTFLYSRELRWFAYWGQGTLVTVSS

SEQ ID NO: 68 - protein, 123 aa, synthetic construct
  REGION 1..123: note = VH of K1G5, K2G5, K3G5, K4G5
QVQLVQSGAEVKKPGATVKISCKVSGDTITAYYMHWVRQAPGQGLEWIGRIDPEDDSTKYAENFKGRVTITADTSTDTAYMELSSLRSEDTAVYYCTTVTFYYTRELRWFAYWGQGTLVTVSS

SEQ ID NO: 69 - protein, 123 aa, synthetic construct
  REGION 1..123: note = VH of K1G6, K2G6, K3G6, K4G6
QVQLVQSGAEVKKPGATVKISCKVSGDTITAYYMHWVRQAPGQGLEWIGRIDPDDDSTKYAENFKGRVTITADTSTDTAYMELSSLRSEDTAVYYCTTITFYYSRELRWFAYWGQGTLVTVSS

SEQ ID NO: 70 - protein, 123 aa, synthetic construct
  REGION 1..123: note = VH of K1G7, K2G7, K3G7, K4G7
QVQLVQSGAEVKKPGATVKISCKVSGDTITAYYMHWVRQAPGQGLEWIGRIDPEDDSTKYAENFKGRVTITADTSTDTAYMELSSLRSEDTAVYYCTTITFYYTRELRWFAYWGQGTLVTVSS

SEQ ID NO: 71 - protein, 123 aa, synthetic construct
  REGION 1..123: note = VH of K1G8, K2G8, K3G8, K4G8
QVQLVQSGAEVKKPGATVKISCKVSGDTITAYYMHWVRQAPGQGLEWIGRIDPEDDSTKYAENFKGRVTITADTSTDTAYMELSSLRSEDTAVYYCTTITFLYSRELRWFAYWGQGTLVTVSS

SEQ ID NO: 72 - protein, 123 aa, synthetic construct
  REGION 1..123: note = VH of K1G9, K2G9, K3G9, K4G9
QVQLVQSGAEVKKPGATVKISCKVSGDTITAYYMHWVRQAPGQGLEWIGRIDPEDDSTKYAENFKGRVTITADTSTDTAYMELSSLRSEDTAVYYCTTITFLYTRELRWFAYWGQGTLVTVSS

SEQ ID NO: 73 - protein, 123 aa, synthetic construct
  REGION 1..123: note = VH of K1G10, K2G10, K3G10, K4G10
QVQLVQSGAEVKKPGATVKISCKVSGDTITAYYMHWVRQAPGQGLEWIGRIDPDDDSTKYAENFKGRVTITADTSTDTAYMELSSLRSEDTAVYYCTTITFYYTRELRWFAYWGQGTLVTVSS

SEQ ID NO: 74 - protein, 123 aa, synthetic construct
  REGION 1..123: note = VH of K1G11, K2G11, K3G11, K4G11, and K2G11-Cy01 to K2G11-Cy06, K2G11-Cy09, K2G11-Cy11, and K2G11-Cy12
QVQLVQSGAEVKKPGATVKISCKVSGDTITAYYMHWVRQAPGQGLEWIGRIDPDDDSTKYAENFKGRVTITADTSTDTAYMELSSLRSEDTAVYYCTTITFLYSRELRWFAYWGQGTLVTVSS

SEQ ID NO: 75 - protein, 123 aa, synthetic construct
  REGION 1..123: note = VH of K1G12, K2G12, K3G12, K4G12
QVQLVQSGAEVKKPGATVKISCKVSGDTITAYYMHWVRQAPGQGLEWIGRIDPDDDSTKYAENFKGRVTITADTSTDTAYMELSSLRSEDTAVYYCTTITFLYTRELRWFAYWGQGTLVTVSS

SEQ ID NO: 76 - protein, 107 aa, synthetic construct
  REGION 1..107: note = VL of K1G1 to K1G12
DIVLTQSPATLSLSPGERATLSCQASQYISNYLSWYQQKPGQAPRLLIYQATSLASGIPARFSGSRSGTDFTLTISSLEPEDFAVYYCLQHYSTPYTFGQGTKLEIK

SEQ ID NO: 77 - protein, 107 aa, synthetic construct
  REGION 1..107: note = VL of K2G1 to K2G12, and K2G11-Cy07, K2G11-Cy08, and K2G11-Cy10
DIVLTQSPATLSLSPGERATLSCQASQYISNYLSWYQQKPGQAPRLLIYSATSLASGIPARFSGSRSGTDFTLTISSLEPEDFAVYYCLQHYSTPYTFGQGTKLEIK

SEQ ID NO: 78 - protein, 107 aa, synthetic construct
  REGION 1..107: note = VL of K3G1 to K3G12
DIVLTQSPATLSLSPGERATLSCQASQYIGNYLSWYQQKPGQAPRLLIYQATSLASGIPARFSGSRSGTDFTLTISSLEPEDFAVYYCLQHYSTPYTFGQGTKLEIK

SEQ ID NO: 79 - protein, 107 aa, synthetic construct
  REGION 1..107: note = VL of K4G1 to K4G12
DIVLTQSPATLSLSPGERATLSCQASQYIGNYLSWYQQKPGQAPRLLIYSATSLASGIPARFSGSRSGTDFTLTISSLEPEDFAVYYCLQHYSTPYTFGQGTKLEIK

SEQ ID NO: 80 - protein, 107 aa, synthetic construct
  REGION 1..107: note = VL of H6K3(H)-Cy01
DIVLTQSPATLSLSPGERATLSCQASQDICNYLSWYQQKPGQAPRLLIYSATSLASGIPARFSGSRSGTDFTLTISSLEPEDFAVYYCLQHYSTPYTFGQGTKLEIK

SEQ ID NO: 81 - protein, 107 aa, synthetic construct
  REGION 1..107: note = VL of H6K3(H)-Cy02
DIVLTQSPATLSLSPGERATLSCQASQDIGCYLSWYQQKPGQAPRLLIYSATSLASGIPARFSGSRSGTDFTLTISSLEPEDFAVYYCLQHYSTPYTFGQGTKLEIK

SEQ ID NO: 82 - protein, 107 aa, synthetic construct
  REGION 1..107: note = VL of H6K3(H)-Cy03
DIVLTQSPATLSLSPGERATLSCQASQDIGNYLSWYQQKPGQAPRLLIYCATSLASGIPARFSGSRSGTDFTLTISSLEPEDFAVYYCLQHYSTPYTFGQGTKLEIK

SEQ ID NO: 83 - protein, 107 aa, synthetic construct
  REGION 1..107: note = VL of H6K3(H)-Cy04
DIVLTQSPATLSLSPGERATLSCQASQDIGNYLSWYQQKPGQAPRLLIYSACSLASGIPARFSGSRSGTDFTLTISSLEPEDFAVYYCLQHYSTPYTFGQGTKLEIK

SEQ ID NO: 84 - protein, 107 aa, synthetic construct
  REGION 1..107: note = VL of H6K3(H)-Cy05
DIVLTQSPATLSLSPGERATLSCQASQDIGNYLSWYQQKPGQAPRLLIYSATSLASGIPARFSGSRCGTDFTLTISSLEPEDFAVYYCLQHYSTPYTFGQGTKLEIK

SEQ ID NO: 85 - protein, 107 aa, synthetic construct
  REGION 1..107: note = VL of H6K3(H)-Cy06
DIVLTQSPATLSLSPGERATLSCQASQDIGNYLSWYQQKPGQAPRLLIYSATSLASGIPARFSGSRSCTDFTLTISSLEPEDFAVYYCLQHYSTPYTFGQGTKLEIK

SEQ ID NO: 86 - protein, 123 aa, synthetic construct
  REGION 1..123: note = VH of H6K3(H)-Cy07, H6K3(H)-Cy08, H6K3(H)-Cy10, and Each Mutant of H6K3(H)-Cy08
QVQLVQSGAEVKKPGATVKISCKVSGDTITAYYMHWVRQAPGQGLEWIGRIDPEDDSTKYAENFKGRVTITADTSTDTAYMELSSLRSEDTAVYYCTTVTCYYSRELRWFAYWGQGTLVTVSS

SEQ ID NO: 87 - protein, 107 aa, synthetic construct
  REGION 1..107: note = VL of H6K3(H)-Cy08-DE
EIVLTQSPATLSLSPGERATLSCQASQDIGNYLSWYQQKPGQAPRLLIYSATSLASGIPARFSGSRSGTDFTLTISSLEPEDFAVYYCLQHYSTPYTFGQGTKLEIK

SEQ ID NO: 88 - protein, 107 aa, synthetic construct
  REGION 1..107: note = VL of H6K3(H)-Cy08-QD
DIVLTQSPATLSLSPGERATLSCQASDDIGNYLSWYQQKPGQAPRLLIYSATSLASGIPARFSGSRSGTDFTLTISSLEPEDFAVYYCLQHYSTPYTFGQGTKLEIK

SEQ ID NO: 89 - protein, 107 aa, synthetic construct
  REGION 1..107: note = VL of H6K3(H)-Cy08-QE
DIVLTQSPATLSLSPGERATLSCQASEDIGNYLSWYQQKPGQAPRLLIYSATSLASGIPARFSGSRSGTDFTLTISSLEPEDFAVYYCLQHYSTPYTFGQGTKLEIK

SEQ ID NO: 90 - protein, 107 aa, synthetic construct
  REGION 1..107: note = VL of H6K3(H)-Cy08-QS
DIVLTQSPATLSLSPGERATLSCQASSDIGNYLSWYQQKPGQAPRLLIYSATSLASGIPARFSGSRSGTDFTLTISSLEPEDFAVYYCLQHYSTPYTFGQGTKLEIK

SEQ ID NO: 91 - protein, 107 aa, synthetic construct
  REGION 1..107: note = VL of H6K3(H)-Cy08-QG
DIVLTQSPATLSLSPGERATLSCQASGDIGNYLSWYQQKPGQAPRLLIYSATSLASGIPARFSGSRSGTDFTLTISSLEPEDFAVYYCLQHYSTPYTFGQGTKLEIK

SEQ ID NO: 92 - protein, 107 aa, synthetic construct
  REGION 1..107: note = VL of H6K3(H)-Cy08-QK
DIVLTQSPATLSLSPGERATLSCQASKDIGNYLSWYQQKPGQAPRLLIYSATSLASGIPARFSGSRSGTDFTLTISSLEPEDFAVYYCLQHYSTPYTFGQGTKLEIK

SEQ ID NO: 93 - protein, 107 aa, synthetic construct
  REGION 1..107: note = VL of H6K3(H)-Cy08-QR
DIVLTQSPATLSLSPGERATLSCQASRDIGNYLSWYQQKPGQAPRLLIYSATSLASGIPARFSGSRSGTDFTLTISSLEPEDFAVYYCLQHYSTPYTFGQGTKLEIK

SEQ ID NO: 94 - protein, 20 aa, synthetic construct
  REGION 1..20: note = linker
GGGGSGGGGSGGGGSGGGGS

SEQ ID NO: 95 - protein, 276 aa, synthetic construct
  REGION 1..276: note = The first polypeptide of H6K3(H)-Cy01
APTSSSTKKTQLQLEHLLLDLQMILNGINNYKNPKLTRMLTFKFYMPKKATELKHLQCLECELGPLEEVLNLAQSKNFHLRPRDLISNIRVIVLELKGSETTFMCEYADETATIVEFLNRWITFCQSIISTLTGGGGSGGGGSGGGGSGGGGSQVQLVQSGAEVKKPGATVKISCKVSGDTITAYYMHWVRQAPGQGLEWIGRIDPEDDSTKYAENFKGRVTITADTSTDTAYMELSSLRSEDTAVYYCTTVTFYYSRELRWFAYWGQGTLVTVSS

SEQ ID NO: 96 - protein, 276 aa, synthetic construct; identical to SEQ ID NO: 95
  REGION 1..276: note = The first polypeptide of H6K3(H)-Cy02

SEQ ID NO: 97 - protein, 276 aa, synthetic construct; identical to SEQ ID NO: 95
  REGION 1..276: note = The first polypeptide of H6K3(H)-Cy03

SEQ ID NO: 98 - protein, 276 aa, synthetic construct
  REGION 1..276: note = The first polypeptide of H6K3(H)-Cy04
APTSSSTKKTQLQLEHLLLDLQMILNGINNYKNPKLTRMLTFKFYMPKKATELKHLQCLEEELGPLEEVLNLAQSKNFHLRPRDLISNIRVIVLELKGSETTFCCEYADETATIVEFLNRWITFCQSIISTLTGGGGSGGGGSGGGGSGGGGSQVQLVQSGAEVKKPGATVKISCKVSGDTITAYYMHWVRQAPGQGLEWIGRIDPEDDSTKYAENFKGRVTITADTSTDTAYMELSSLRSEDTAVYYCTTVTFYYSRELRWFAYWGQGTLVTVSS

SEQ ID NO: 99 - protein, 276 aa, synthetic construct
  REGION 1..276: note = The first polypeptide of H6K3(H)-Cy05
APTSSSTKKTQLQLEHLLLDLQMILNGINNYKNPKLTRMLTFKFYMPKKATELKHLQCLEEELGPLEEVLNLAQSKNFHLRPRDLISNIRVIVLELKGSETCFMCEYADETATIVEFLNRWITFCQSIISTLTGGGGSGGGGSGGGGSGGGGSQVQLVQSGAEVKKPGATVKISCKVSGDTITAYYMHWVRQAPGQGLEWIGRIDPEDDSTKYAENFKGRVTITADTSTDTAYMELSSLRSEDTAVYYCTTVTFYYSRELRWFAYWGQGTLVTVSS

SEQ ID NO: 100 - protein, 276 aa, synthetic construct; identical to SEQ ID NO: 99
  REGION 1..276: note = The first polypeptide of H6K3(H)-Cy06

SEQ ID NO: 101 - protein, 276 aa, synthetic construct
  REGION 1..276: note = The first polypeptide of H6K3(H)-Cy07
APTSSSTKKTQLQLEHLLLDLQMILNGINNYKNPKLTRMLTFKFYMPKKATELKHLQCLEEELCPLEEVLNLAQSKNFHLRPRDLISNIRVIVLELKGSETTFMCEYADETATIVEFLNRWITFCQSIISTLTGGGGSGGGGSGGGGSGGGGSQVQLVQSGAEVKKPGATVKISCKVSGDTITAYYMHWVRQAPGQGLEWIGRIDPEDDSTKYAENFKGRVTITADTSTDTAYMELSSLRSEDTAVYYCTTVTCYYSRELRWFAYWGQGTLVTVSS

SEQ ID NO: 102 - protein, 276 aa, synthetic construct
  REGION 1..276: note = The first polypeptide of H6K3(H)-Cy08
APTSSSTKKTQLQLEHLLLDLQMILNGINNYKNPKLTRMLTFKFYMPKKATELKHLQCLEEELGCLEEVLNLAQSKNFHLRPRDLISNIRVIVLELKGSETTFMCEYADETATIVEFLNRWITFCQSIISTLTGGGGSGGGGSGGGGSGGGGSQVQLVQSGAEVKKPGATVKISCKVSGDTITAYYMHWVRQAPGQGLEWIGRIDPEDDSTKYAENFKGRVTITADTSTDTAYMELSSLRSEDTAVYYCTTVTCYYSRELRWFAYWGQGTLVTVSS

SEQ ID NO: 103 - protein, 273 aa, synthetic construct
  REGION 1..273: note = The first polypeptide of H6K3(H)-Cy10
SSSTKKTQLQLEHLLLDLQMILNGINNYKNPKLTRMLTCKFYMPKKATELKHLQCLEEELGPLEEVLNLAQSKNFHLRPRDLISNIRVIVLELKGSETTFMCEYADETATIVEFLNRWITFLQSIISTLTGGGGSGGGGSGGGGSGGGGSQVQLVQSGAEVKKPGATVKISCKVSGDTITAYYMHWVRQAPGQGLEWIGRIDPEDDSTKYAENFKGRVTITADTSTDTAYMELSSLRSEDTAVYYCTTVTCYYSRELRWFAYWGQGTLVTVSS

SEQ ID NO: 104 - protein, 107 aa, synthetic construct
  REGION 1..107: note = VL of K2G11-Cy01,and K2G11-Cy11
DIVLTQSPATLSLSPGERATLSCQASQYICNYLSWYQQKPGQAPRLLIYSATSLASGIPARFSGSRSGTDFTLTISSLEPEDFAVYYCLQHYSTPYTFGQGTKLEIK

SEQ ID NO: 105 - protein, 107 aa, synthetic construct
  REGION 1..107: note = VL of K2G11-Cy02
DIVLTQSPATLSLSPGERATLSCQASQYISCYLSWYQQKPGQAPRLLIYSATSLASGIPARFSGSRSGTDFTLTISSLEPEDFAVYYCLQHYSTPYTFGQGTKLEIK

SEQ ID NO: 106 - protein, 107 aa, synthetic construct
  REGION 1..107: note = VL of K2G11-Cy03
DIVLTQSPATLSLSPGERATLSCQASQYISNYLSWYQQKPGQAPRLLIYCATSLASGIPARFSGSRSGTDFTLTISSLEPEDFAVYYCLQHYSTPYTFGQGTKLEIK

SEQ ID NO: 107 - protein, 107 aa, synthetic construct
  REGION 1..107: note = VL of K2G11-Cy04
DIVLTQSPATLSLSPGERATLSCQASQYISNYLSWYQQKPGQAPRLLIYSACSLASGIPARFSGSRSGTDFTLTISSLEPEDFAVYYCLQHYSTPYTFGQGTKLEIK

SEQ ID NO: 108 - protein, 107 aa, synthetic construct
  REGION 1..107: note = VL of K2G11-Cy05
DIVLTQSPATLSLSPGERATLSCQASQYISNYLSWYQQKPGQAPRLLIYSATSLASGIPARFSGSRCGTDFTLTISSLEPEDFAVYYCLQHYSTPYTFGQGTKLEIK

SEQ ID NO: 109 - protein, 107 aa, synthetic construct
  REGION 1..107: note = VL of K2G11-Cy06
DIVLTQSPATLSLSPGERATLSCQASQYISNYLSWYQQKPGQAPRLLIYSATSLASGIPARFSGSRSCTDFTLTISSLEPEDFAVYYCLQHYSTPYTFGQGTKLEIK

SEQ ID NO: 110 - protein, 107 aa, synthetic construct
  REGION 1..107: note = VL of K2G11-Cy09
DIVLTQSPATLSLSPGERATLSCQASQYISNYLSWYQQKPGQAPRLLIYSATSLASGIPARFSGSRSGTDFTLTISSLEPEDFAVYYCLQHCSTPYTFGQGTKLEIK

SEQ ID NO: 111 - protein, 107 aa, synthetic construct
  REGION 1..107: note = VL of K2G11-Cy12
DIVLTQSPATLSLSPGERATLSCQASQYISNCLSWYQQKPGQAPRLLIYSATSLASGIPARFSGSRSGTDFTLTISSLEPEDFAVYYCLQHYSTPYTFGQGTKLEIK

SEQ ID NO: 112 - protein, 123 aa, synthetic construct
  REGION 1..123: note = VH of K2G11-Cy07, K2G11-Cy08, and K2G11-Cy10
QVQLVQSGAEVKKPGATVKISCKVSGDTITAYYMHWVRQAPGQGLEWIGRIDPDDDSTKYAENFKGRVTITADTSTDTAYMELSSLRSEDTAVYYCTTITCLYSRELRWFAYWGQGTLVTVSS

SEQ ID NO: 113 - protein, 273 aa, synthetic construct
  REGION 1..273: note = The first polypeptide of K2G11-Cy01, K2G11-Cy02, and K2G11-Cy03
SSSTKKTQLQLEHLLLDLQMILNGINNYKNPKLTRMLTFKFYMPKKATELKHLQCLECELGPLEEVLNLAQSKNFHLRPRDLISNIRVIVLELKGSETTFMCEYADETATIVEFLNRWITFLQSIISTLTGGGGSGGGGSGGGGSGGGGSQVQLVQSGAEVKKPGATVKISCKVSGDTITAYYMHWVRQAPGQGLEWIGRIDPDDDSTKYAENFKGRVTITADTSTDTAYMELSSLRSEDTAVYYCTTITFLYSRELRWFAYWGQGTLVTVSS

SEQ ID NO: 114 - protein, 273 aa, synthetic construct
  REGION 1..273: note = The first polypeptide of K2G11-Cy04
SSSTKKTQLQLEHLLLDLQMILNGINNYKNPKLTRMLTFKFYMPKKATELKHLQCLEEELGPLEEVLNLAQSKNFHLRPRDLISNIRVIVLELKGSETTFCCEYADETATIVEFLNRWITFLQSIISTLTGGGGSGGGGSGGGGSGGGGSQVQLVQSGAEVKKPGATVKISCKVSGDTITAYYMHWVRQAPGQGLEWIGRIDPDDDSTKYAENFKGRVTITADTSTDTAYMELSSLRSEDTAVYYCTTITFLYSRELRWFAYWGQGTLVTVSS

SEQ ID NO: 115 - protein, 273 aa, synthetic construct
  REGION 1..273: note = The first polypeptide of K2G11-Cy05 and K2G11-Cy06
SSSTKKTQLQLEHLLLDLQMILNGINNYKNPKLTRMLTFKFYMPKKATELKHLQCLEEELGPLEEVLNLAQSKNFHLRPRDLISNIRVIVLELKGSETCFMCEYADETATIVEFLNRWITFLQSIISTLTGGGGSGGGGSGGGGSGGGGSQVQLVQSGAEVKKPGATVKISCKVSGDTITAYYMHWVRQAPGQGLEWIGRIDPDDDSTKYAENFKGRVTITADTSTDTAYMELSSLRSEDTAVYYCTTITFLYSRELRWFAYWGQGTLVTVSS

SEQ ID NO: 116 - protein, 273 aa, synthetic construct
  REGION 1..273: note = The first polypeptide of K2G11-Cy07
SSSTKKTQLQLEHLLLDLQMILNGINNYKNPKLTRMLTFKFYMPKKATELKHLQCLEEELCPLEEVLNLAQSKNFHLRPRDLISNIRVIVLELKGSETTFMCEYADETATIVEFLNRWITFLQSIISTLTGGGGSGGGGSGGGGSGGGGSQVQLVQSGAEVKKPGATVKISCKVSGDTITAYYMHWVRQAPGQGLEWIGRIDPDDDSTKYAENFKGRVTITADTSTDTAYMELSSLRSEDTAVYYCTTITCLYSRELRWFAYWGQGTLVTVSS

SEQ ID NO: 117 - protein, 273 aa, synthetic construct
  REGION 1..273: note = The first polypeptide of K2G11-Cy08
SSSTKKTQLQLEHLLLDLQMILNGINNYKNPKLTRMLTFKFYMPKKATELKHLQCLEEELGCLEEVLNLAQSKNFHLRPRDLISNIRVIVLELKGSETTFMCEYADETATIVEFLNRWITFLQSIISTLTGGGGSGGGGSGGGGSGGGGSQVQLVQSGAEVKKPGATVKISCKVSGDTITAYYMHWVRQAPGQGLEWIGRIDPDDDSTKYAENFKGRVTITADTSTDTAYMELSSLRSEDTAVYYCTTITCLYSRELRWFAYWGQGTLVTVSS

SEQ ID NO: 118 - protein, 273 aa, synthetic construct
  REGION 1..273: note = The first polypeptide of K2G11-Cy09 and K2G11-Cy12
SSSTKKTQLQLEHLLLDLQMILNGINNYKNPKLTRMLTFKFYMPKKATELKHLQCLEEELCPLEEVLNLAQSKNFHLRPRDLISNIRVIVLELKGSETTFMCEYADETATIVEFLNRWITFLQSIISTLTGGGGSGGGGSGGGGSGGGGSQVQLVQSGAEVKKPGATVKISCKVSGDTITAYYMHWVRQAPGQGLEWIGRIDPDDDSTKYAENFKGRVTITADTSTDTAYMELSSLRSEDTAVYYCTTITFLYSRELRWFAYWGQGTLVTVSS

SEQ ID NO: 119 - protein, 273 aa, synthetic construct
  REGION 1..273: note = The first polypeptide of K2G11-Cy10
SSSTKKTQLQLEHLLLDLQMILNGINNYKNPKLTRMLTCKFYMPKKATELKHLQCLEEELGPLEEVLNLAQSKNFHLRPRDLISNIRVIVLELKGSETTFMCEYADETATIVEFLNRWITFLQSIISTLTGGGGSGGGGSGGGGSGGGGSQVQLVQSGAEVKKPGATVKISCKVSGDTITAYYMHWVRQAPGQGLEWIGRIDPDDDSTKYAENFKGRVTITADTSTDTAYMELSSLRSEDTAVYYCTTITCLYSRELRWFAYWGQGTLVTVSS

SEQ ID NO: 120 - protein, 273 aa, synthetic construct
  REGION 1..273: note = The first polypeptide of K2G11-Cy11
SSSTKKTQLQLEHLLLDLQMILNGINNYKNPKLTRMLTFKFYMPKKATELKHLQCLCEELGPLEEVLNLAQSKNFHLRPRDLISNIRVIVLELKGSETTFMCEYADETATIVEFLNRWITFLQSIISTLTGGGGSGGGGSGGGGSGGGGSQVQLVQSGAEVKKPGATVKISCKVSGDTITAYYMHWVRQAPGQGLEWIGRIDPDDDSTKYAENFKGRVTITADTSTDTAYMELSSLRSEDTAVYYCTTITFLYSRELRWFAYWGQGTLVTVSS

SEQ ID NO: 121 - protein, 133 aa, synthetic construct
  REGION 1..133: note = hIL-2 mutant (hIL2-DM) introdued with the amino acid mutation E61C
APTSSSTKKTQLQLEHLLLDLQMILNGINNYKNPKLTRMLTFKFYMPKKATELKHLQCLECELGPLEEVLNLAQSKNFHLRPRDLISNIRVIVLELKGSETTFMCEYADETATIVEFLNRWITFCQSIISTLT

SEQ ID NO: 122 - protein, 133 aa, synthetic construct
  REGION 1..133: note = hIL-2 mutant (hIL2-DM) introdued with the amino acid mutation M104C
APTSSSTKKTQLQLEHLLLDLQMILNGINNYKNPKLTRMLTFKFYMPKKATELKHLQCLEEELGPLEEVLNLAQSKNFHLRPRDLISNIRVIVLELKGSETTFCCEYADETATIVEFLNRWITFCQSIISTLT

SEQ ID NO: 123 - protein, 133 aa, synthetic construct
  REGION 1..133: note = hIL-2 mutant (hIL2-DM) introdued with the amino acid mutation T102C
APTSSSTKKTQLQLEHLLLDLQMILNGINNYKNPKLTRMLTFKFYMPKKATELKHLQCLEEELGPLEEVLNLAQSKNFHLRPRDLISNIRVIVLELKGSETCFMCEYADETATIVEFLNRWITFCQSIISTLT

SEQ ID NO: 124 - protein, 133 aa, synthetic construct
  REGION 1..133: note = hIL-2 mutant (hIL2-DM) introdued with the amino acid mutation K64C
APTSSSTKKTQLQLEHLLLDLQMILNGINNYKNPKLTRMLTFKFYMPKKATELKHLQCLEEELCPLEEVLNLAQSKNFHLRPRDLISNIRVIVLELKGSETTFMCEYADETATIVEFLNRWITFCQSIISTLT

SEQ ID NO: 125 - protein, 133 aa, synthetic construct
  REGION 1..133: note = hIL-2 mutant (hIL2-DM) introdued with the amino acid mutation P65C
APTSSSTKKTQLQLEHLLLDLQMILNGINNYKNPKLTRMLTFKFYMPKKATELKHLQCLEEELGCLEEVLNLAQSKNFHLRPRDLISNIRVIVLELKGSETTFMCEYADETATIVEFLNRWITFCQSIISTLT

SEQ ID NO: 126 - protein, 130 aa, synthetic construct
  REGION 1..130: note = hIL-2 mutant (hIL2-DM) in which Cys substitution E61C is introduced, and the first 3 amino acids of N-terminal are deleted and the amino acid mutation C125L is introduced
SSSTKKTQLQLEHLLLDLQMILNGINNYKNPKLTRMLTFKFYMPKKATELKHLQCLECELGPLEEVLNLAQSKNFHLRPRDLISNIRVIVLELKGSETTFMCEYADETATIVEFLNRWITFLQSIISTLT

SEQ ID NO: 127 - protein, 130 aa, synthetic construct
  REGION 1..130: note = hIL-2 mutant (hIL2-DM) in which Cys substitution M104C is introduced, and the first 3 amino acids of N-terminal are deleted and the amino acid mutation C125L is introduced
SSSTKKTQLQLEHLLLDLQMILNGINNYKNPKLTRMLTFKFYMPKKATELKHLQCLEEELGPLEEVLNLAQSKNFHLRPRDLISNIRVIVLELKGSETTFCCEYADETATIVEFLNRWITFLQSIISTLT

SEQ ID NO: 128 - protein, 130 aa, synthetic construct
  REGION 1..130: note = hIL-2 mutant (hIL2-DM) in which Cys substitution T102C is introduced, and the first 3 amino acids of N-terminal are deleted and the amino acid mutation C125L is introduced
SSSTKKTQLQLEHLLLDLQMILNGINNYKNPKLTRMLTFKFYMPKKATELKHLQCLEEELGPLEEVLNLAQSKNFHLRPRDLISNIRVIVLELKGSETCFMCEYADETATIVEFLNRWITFLQSIISTLT

SEQ ID NO: 129 - protein, 130 aa, synthetic construct
  REGION 1..130: note = hIL-2 mutant (hIL2-DM) in which Cys substitution K64C is introduced, and the first 3 amino acids of N-terminal are deleted and the amino acid mutation C125L is introduced
SSSTKKTQLQLEHLLLDLQMILNGINNYKNPKLTRMLTFKFYMPKKATELKHLQCLEEELCPLEEVLNLAQSKNFHLRPRDLISNIRVIVLELKGSETTFMCEYADETATIVEFLNRWITFLQSIISTLT

SEQ ID NO: 130 - protein, 130 aa, synthetic construct
  REGION 1..130: note = hIL-2 mutant (hIL2-DM) in which Cys substitution P65C is introduced, and the first 3 amino acids of N-terminal are deleted and the amino acid mutation C125L is introduced
SSSTKKTQLQLEHLLLDLQMILNGINNYKNPKLTRMLTFKFYMPKKATELKHLQCLEEELGCLEEVLNLAQSKNFHLRPRDLISNIRVIVLELKGSETTFMCEYADETATIVEFLNRWITFLQSIISTLT

SEQ ID NO: 131 - protein, 130 aa, synthetic construct
  REGION 1..130: note = hIL-2 mutant (hIL2-DM) in which Cys substitution F42C is introduced, and the first 3 amino acids of N-terminal are deleted and the amino acid mutation C125L is introduced
SSSTKKTQLQLEHLLLDLQMILNGINNYKNPKLTRMLTCKFYMPKKATELKHLQCLEEELGPLEEVLNLAQSKNFHLRPRDLISNIRVIVLELKGSETTFMCEYADETATIVEFLNRWITFLQSIISTLT

SEQ ID NO: 132 - protein, 130 aa, synthetic construct
  REGION 1..130: note = hIL-2 mutant (hIL2-DM) in which Cys substitution E60C is introduced, and the first 3 amino acids of N-terminal are deleted and the amino acid mutation C125L is introduced
SSSTKKTQLQLEHLLLDLQMILNGINNYKNPKLTRMLTFKFYMPKKATELKHLQCLCEELGPLEEVLNLAQSKNFHLRPRDLISNIRVIVLELKGSETTFMCEYADETATIVEFLNRWITFLQSIISTLT

SEQ ID NO: 133 - protein, 273 aa, synthetic construct
  REGION 1..273: note = The first polypeptide of IC-Cy08 (delta 3, WT)
SSSTKKTQLQLEHLLLDLQMILNGINNYKNPKLTRMLTFKFYMPKKATELKHLQCLEEELGCLEEVLNLAQSKNFHLRPRDLISNIRVIVLELKGSETTFMCEYADETATIVEFLNRWITFCQSIISTLTGGGGSGGGGSGGGGSGGGGSQVQLVQSGAEVKKPGATVKISCKVSGDTITAYYMHWVRQAPGQGLEWIGRIDPEDDSTKYAENFKGRVTITADTSTDTAYMELSSLRSEDTAVYYCTTVTCYYSRELRWFAYWGQGTLVTVSS

SEQ ID NO: 134 - protein, 273 aa, synthetic construct
  REGION 1..273: note = The first polypeptide of IC-Cy08 (delta 3, C125A)
SSSTKKTQLQLEHLLLDLQMILNGINNYKNPKLTRMLTFKFYMPKKATELKHLQCLEEELGCLEEVLNLAQSKNFHLRPRDLISNIRVIVLELKGSETTFMCEYADETATIVEFLNRWITFAQSIISTLTGGGGSGGGGSGGGGSGGGGSQVQLVQSGAEVKKPGATVKISCKVSGDTITAYYMHWVRQAPGQGLEWIGRIDPEDDSTKYAENFKGRVTITADTSTDTAYMELSSLRSEDTAVYYCTTVTCYYSRELRWFAYWGQGTLVTVSS

SEQ ID NO: 135 - protein, 273 aa, synthetic construct
  REGION 1..273: note = The first polypeptide of IC-Cy08 (delta 3, C125L)
SSSTKKTQLQLEHLLLDLQMILNGINNYKNPKLTRMLTFKFYMPKKATELKHLQCLEEELGCLEEVLNLAQSKNFHLRPRDLISNIRVIVLELKGSETTFMCEYADETATIVEFLNRWITFLQSIISTLTGGGGSGGGGSGGGGSGGGGSQVQLVQSGAEVKKPGATVKISCKVSGDTITAYYMHWVRQAPGQGLEWIGRIDPEDDSTKYAENFKGRVTITADTSTDTAYMELSSLRSEDTAVYYCTTVTCYYSRELRWFAYWGQGTLVTVSS

SEQ ID NO: 136 - protein, 273 aa, synthetic construct
  REGION 1..273: note = The first polypeptide of IC-Cy08 (delta 3, C125S)
SSSTKKTQLQLEHLLLDLQMILNGINNYKNPKLTRMLTFKFYMPKKATELKHLQCLEEELGCLEEVLNLAQSKNFHLRPRDLISNIRVIVLELKGSETTFMCEYADETATIVEFLNRWITFSQSIISTLTGGGGSGGGGSGGGGSGGGGSQVQLVQSGAEVKKPGATVKISCKVSGDTITAYYMHWVRQAPGQGLEWIGRIDPEDDSTKYAENFKGRVTITADTSTDTAYMELSSLRSEDTAVYYCTTVTCYYSRELRWFAYWGQGTLVTVSS

SEQ ID NO: 137 - protein, 273 aa, synthetic construct
  REGION 1..273: note = The first polypeptide of IC-Cy08 (delta 3, C125Q)
SSSTKKTQLQLEHLLLDLQMILNGINNYKNPKLTRMLTFKFYMPKKATELKHLQCLEEELGCLEEVLNLAQSKNFHLRPRDLISNIRVIVLELKGSETTFMCEYADETATIVEFLNRWITFQQSIISTLTGGGGSGGGGSGGGGSGGGGSQVQLVQSGAEVKKPGATVKISCKVSGDTITAYYMHWVRQAPGQGLEWIGRIDPEDDSTKYAENFKGRVTITADTSTDTAYMELSSLRSEDTAVYYCTTVTCYYSRELRWFAYWGQGTLVTVSS

SEQ ID NO: 138 - protein, 273 aa, synthetic construct
  REGION 1..273: note = The first polypeptide of IC-Cy08 (delta 3, C125V)
SSSTKKTQLQLEHLLLDLQMILNGINNYKNPKLTRMLTFKFYMPKKATELKHLQCLEEELGCLEEVLNLAQSKNFHLRPRDLISNIRVIVLELKGSETTFMCEYADETATIVEFLNRWITFVQSIISTLTGGGGSGGGGSGGGGSGGGGSQVQLVQSGAEVKKPGATVKISCKVSGDTITAYYMHWVRQAPGQGLEWIGRIDPEDDSTKYAENFKGRVTITADTSTDTAYMELSSLRSEDTAVYYCTTVTCYYSRELRWFAYWGQGTLVTVSS

SEQ ID NO: 139 - protein, 130 aa, synthetic construct
  REGION 1..130: note = hIL2-DM(delta 3, C125L)
SSSTKKTQLQLEHLLLDLQMILNGINNYKNPKLTRMLTFKFYMPKKATELKHLQCLEEELGPLEEVLNLAQSKNFHLRPRDLISNIRVIVLELKGSETTFMCEYADETATIVEFLNRWITFLQSIISTLT

SEQ ID NO: 140 - protein, 121 aa, synthetic construct [sequence omitted]

SEQ ID NO: 141 - protein, 111 aa, synthetic construct
  REGION 1..111: note = VL of NARA1, NARA1-Cy01 to NARA1-Cy03, NARA1-Cy09 to NARA1-Cy11
DIVLTQSPASLAVSLGQRATISCKASQSVDYDGDSYMNWYQQKPGQPPKLLIYAASNLESGIPARFSGSGSGTDFTLNIHPVEEEDAATYYCQQSNEDPYTFGGGTKLEIK

SEQ ID NO: 142 - protein, 5 aa, synthetic construct
  REGION 1..5: note = HCDR1 of NARA1, NARA1-Cy01 to NARA1-Cy08, NARA1-Cy10, NARA1-Cy11
NYLIE

SEQ ID NO: 143 - protein, 17 aa, synthetic construct
  REGION 1..17: note = HCDR2 of NARA1, NARA1-Cy02 to NARA1-Cy09
VINPGSGGTNYNEKFKG

SEQ ID NO: 144 - protein, 12 aa, synthetic construct
  REGION 1..12: note = HCDR3 of NARA1, NARA1-Cy01, NARA1-Cy04 to NARA1-Cy11
WRGDGYYAYFDV

SEQ ID NO: 145 - protein, 15 aa, synthetic construct
  REGION 1..15: note = LCDR1 of NARA1, NARA1-Cy01 to NARA1-Cy03, NARA1-Cy06 to NARA1-Cy11
KASQSVDYDGDSYMN

SEQ ID NO: 146 - protein, 7 aa, synthetic construct
  REGION 1..7: note = LCDR2 of NARA1, NARA1-Cy01 to NARA1-Cy11
AASNLES

SEQ ID NO: 147 - protein, 9 aa, synthetic construct
  REGION 1..9: note = HCDR1 of NARA1-Cy09
QQSNEDPYT

SEQ ID NO: 148 - protein, 5 aa, synthetic construct
  REGION 1..5: note = HCDR1
CYLIE

SEQ ID NO: 149 - protein, 17 aa, synthetic construct
  REGION 1..17: note = HCDR2 of NARA1-Cy01
VINPGCGGTNYNEKFKG

SEQ ID NO: 150 - protein, 17 aa, synthetic construct
  REGION 1..17: note = HCDR2 of NARA1-Cy10
VCNPGSGGTNYNEKFKG

SEQ ID NO: 151 - protein, 17 aa, synthetic construct
  REGION 1..17: note = HCDR2 of NARA1-Cy11
VINPGSGCTNYNEKFKG

SEQ ID NO: 152 - protein, 12 aa, synthetic construct
  REGION 1..12: note = HCDR3 of NARA1-Cy02
WRCDGYYAYFDV

SEQ ID NO: 153 - protein, 12 aa, synthetic construct
  REGION 1..12: note = HCDR3 of NARA1-Cy03
WRGDGYYCYFDV

SEQ ID NO: 154 - protein, 15 aa, synthetic construct
  REGION 1..15: note = LCDR1 of NARA1-Cy04 and NARA1-Cy05
KASQSVDYCGDSYMN

SEQ ID NO: 155 - protein, 9 aa, synthetic construct
  REGION 1..9: note = LCDR3 of NARA1-Cy06
QQCNEDPYT

SEQ ID NO: 156 - protein, 9 aa, synthetic construct
  REGION 1..9: note = LCDR3 of NARA1-Cy07
QQSCEDPYT

SEQ ID NO: 157 - protein, 9 aa, synthetic construct
  REGION 1..9: note = LCDR3 of NARA1-Cy08
QQSNECPYT

SEQ ID NO: 158 - protein, 121 aa, synthetic construct
  REGION 1..121: note = VH of NARA1-Cy01
QVQLQQSGAELVRPGTSVKVSCKASGYAFTNYLIEWVKQRPGQGLEWIGVINPGCGGTNYNEKFKGKATLTADKSSSTAYMQLSSLTSDDSAVYFCARWRGDGYYAYFDVWGAGTTVTVSS

SEQ ID NO: 159 - protein, 121 aa, synthetic construct
  REGION 1..121: note = VH of NARA1-Cy02
QVQLQQSGAELVRPGTSVKVSCKASGYAFTNYLIEWVKQRPGQGLEWIGVINPGSGGTNYNEKFKGKATLTADKSSSTAYMQLSSLTSDDSAVYFCARWRCDGYYAYFDVWGAGTTVTVSS

SEQ ID NO: 160 - protein, 121 aa, synthetic construct
  REGION 1..121: note = VH of NARA1-Cy03
QVQLQQSGAELVRPGTSVKVSCKASGYAFTNYLIEWVKQRPGQGLEWIGVINPGSGGTNYNEKFKGKATLTADKSSSTAYMQLSSLTSDDSAVYFCARWRGDGYYCYFDVWGAGTTVTVSS

SEQ ID NO: 161 - protein, 121 aa, synthetic construct
  REGION 1..121: note = VH of NARA1-Cy09
QVQLQQSGAELVRPGTSVKVSCKASGYAFTCYLIEWVKQRPGQGLEWIGVINPGSGGTNYNEKFKGKATLTADKSSSTAYMQLSSLTSDDSAVYFCARWRGDGYYAYFDVWGAGTTVTVSS

SEQ ID NO: 162 - protein, 121 aa, synthetic construct
  REGION 1..121: note = VH of NARA1-Cy10
QVQLQQSGAELVRPGTSVKVSCKASGYAFTNYLIEWVKQRPGQGLEWIGVCNPGSGGTNYNEKFKGKATLTADKSSSTAYMQLSSLTSDDSAVYFCARWRGDGYYAYFDVWGAGTTVTVSS

SEQ ID NO: 163 - protein, 121 aa, synthetic construct
  REGION 1..121: note = VH of NARA1-Cy11
QVQLQQSGAELVRPGTSVKVSCKASGYAFTNYLIEWVKQRPGQGLEWIGVINPGSGCTNYNEKFKGKATLTADKSSSTAYMQLSSLTSDDSAVYFCARWRGDGYYAYFDVWGAGTTVTVSS

SEQ ID NO: 164 - protein, 111 aa, synthetic construct
  REGION 1..111: note = VL of NARA1-Cy04, NARA1-Cy05
DIVLTQSPASLAVSLGQRATISCKASQSVDYCGDSYMNWYQQKPGQPPKLLIYAASNLESGIPARFSGSGSGTDFTLNIHPVEEEDAATYYCQQSNEDPYTFGGGTKLEIK

SEQ ID NO: 165 - protein, 111 aa, synthetic construct
  REGION 1..111: note = VL of NARA1-Cy06
DIVLTQSPASLAVSLGQRATISCKASQSVDYDGDSYMNWYQQKPGQPPKLLIYAASNLESGIPARFSGSGSGTDFTLNIHPVEEEDAATYYCQQCNEDPYTFGGGTKLEIK

SEQ ID NO: 166 - protein, 111 aa, synthetic construct
  REGION 1..111: note = VL of NARA1-Cy07
DIVLTQSPASLAVSLGQRATISCKASQSVDYDGDSYMNWYQQKPGQPPKLLIYAASNLESGIPARFSGSGSGTDFTLNIHPVEEEDAATYYCQQSCEDPYTFGGGTKLEIK

SEQ ID NO: 167 - protein, 111 aa, synthetic construct
  REGION 1..111: note = VL of NARA1-Cy08
DIVLTQSPASLAVSLGQRATISCKASQSVDYDGDSYMNWYQQKPGQPPKLLIYAASNLESGIPARFSGSGSGTDFTLNIHPVEEEDAATYYCQQSNECPYTFGGGTKLEIK

SEQ ID NO: 168 - protein, 121 aa, synthetic construct
  REGION 1..121: note = VH of TCB2, TCB2-Cy06 to TCB2-Cy11
QVQLVQSGAEVKKPGASVKVSCKASGYTFTTYWIQWVRQAPGQGLEWMGAIYPGDGDTRYIQNFKGRVTMTRDTSTSTVYMELSSLRSEDTAVYYCARSLATRGFYAMDYWGQGTLVTVSS

SEQ ID NO: 169 - protein, 107 aa, synthetic construct
  REGION 1..107: note = VL of TCB2, TCB2-Cy01 to TCB2-Cy05
DIVMTQSPSSLSASVGDRVTIRCITSTDIDDDMNWYQQKPGKAPKLLISEGNTLRPGVPSRFSGSGYGTDFTFTISSLQPEDIADYYCLQSDNLPYTFGGGTKLEIK

SEQ ID NO: 170 - protein, 5 aa, synthetic construct
  REGION 1..5: note = HCDR1 of TCB2, TCB2-Cy01 to TCB2-Cy11
TYWIQ

SEQ ID NO: 171 - protein, 17 aa, synthetic construct
  REGION 1..17: note = HCDR2 of TCB2, TCB2-Cy01 to TCB2-Cy04, TCB2-Cy06 to TCB2-Cy11
AIYPGDGDTRYIQNFKG

SEQ ID NO: 172 - protein, 12 aa, synthetic construct
  REGION 1..12: note = HCDR3 of TCB2, TCB2-Cy05 to TCB2-Cy11
SLATRGFYAMDY

SEQ ID NO: 173 - protein, 11 aa, synthetic construct
  REGION 1..11: note = LCDR1 of TCB2, TCB2-Cy01 to TCB2-Cy05, TCB2-Cy07 to TCB2-Cy11
ITSTDIDDDMN

SEQ ID NO: 174 - protein, 7 aa, synthetic construct
  REGION 1..7: note = LCDR2 of TCB2, TCB2-Cy01 to TCB2-Cy11
EGNTLRP

SEQ ID NO: 175 - protein, 9 aa, synthetic construct
  REGION 1..9: note = LCDR3 of TCB2, TCB2-Cy01 to TCB2-Cy06
LQSDNLPYT

SEQ ID NO: 176 - protein, 17 aa, synthetic construct
  REGION 1..17: note = HCDR2 of TCB2-Cy05
AIYPGCGDTRYIQNFKG

SEQ ID NO: 177 - protein, 12 aa, synthetic construct
  REGION 1..12: note = HCDR3 of TCB2-Cy01
SLCTRGFYAMDY

SEQ ID NO: 178 - protein, 12 aa, synthetic construct
  REGION 1..12: note = HCDR3 of TCB2-Cy02
SLATCGFYAMDY

SEQ ID NO: 179 - protein, 12 aa, synthetic construct
  REGION 1..12: note = HCDR3 of TCB2-Cy03
SLATRCFYAMDY

SEQ ID NO: 180 - protein, 12 aa, synthetic construct
  REGION 1..12: note = HCDR3 of TCB2-Cy04
SLATRGCYAMDY

SEQ ID NO: 181 - protein, 11 aa, synthetic construct
  REGION 1..11: note = LCDR1 of TCB2-Cy06
ITSCDIDDDMN

SEQ ID NO: 182 - protein, 9 aa, synthetic construct
  REGION 1..9: note = LCDR3 of TCB2-Cy07
LQSCNLPYT

SEQ ID NO: 183 - protein, 9 aa, synthetic construct
  REGION 1..9: note = LCDR3 of TCB2-Cy08 to TCB2-Cy10
LQSDCLPYT

SEQ ID NO: 184 - protein, 9 aa, synthetic construct
  REGION 1..9: note = LCDR3 of TCB2-Cy011
LQSDNCPYT

SEQ ID NO: 185 - protein, 121 aa, synthetic construct
  REGION 1..121: note = VH of TCB2-Cy01
QVQLVQSGAEVKKPGASVKVSCKASGYTFTTYWIQWVRQAPGQGLEWMGAIYPGDGDTRYIQNFKGRVTMTRDTSTSTVYMELSSLRSEDTAVYYCARSLCTRGFYAMDYWGQGTLVTVSS

SEQ ID NO: 186 - protein, 121 aa, synthetic construct
  REGION 1..121: note = VH of TCB2-Cy02
QVQLVQSGAEVKKPGASVKVSCKASGYTFTTYWIQWVRQAPGQGLEWMGAIYPGDGDTRYIQNFKGRVTMTRDTSTSTVYMELSSLRSEDTAVYYCARSLATCGFYAMDYWGQGTLVTVSS

SEQ ID NO: 187 - protein, 121 aa, synthetic construct
  REGION 1..121: note = VH of TCB2-Cy03
QVQLVQSGAEVKKPGASVKVSCKASGYTFTTYWIQWVRQAPGQGLEWMGAIYPGDGDTRYIQNFKGRVTMTRDTSTSTVYMELSSLRSEDTAVYYCARSLATRCFYAMDYWGQGTLVTVSS

SEQ ID NO: 188 - protein, 121 aa, synthetic construct
  REGION 1..121: note = VH of TCB2-Cy04
QVQLVQSGAEVKKPGASVKVSCKASGYTFTTYWIQWVRQAPGQGLEWMGAIYPGDGDTRYIQNFKGRVTMTRDTSTSTVYMELSSLRSEDTAVYYCARSLATRGCYAMDYWGQGTLVTVSS

SEQ ID NO: 189 - protein, 121 aa, synthetic construct
  REGION 1..121: note = VH of TCB2-Cy05
QVQLVQSGAEVKKPGASVKVSCKASGYTFTTYWIQWVRQAPGQGLEWMGAIYPGCGDTRYIQNFKGRVTMTRDTSTSTVYMELSSLRSEDTAVYYCARSLATRGFYAMDYWGQGTLVTVSS

SEQ ID NO: 190 - protein, 107 aa, synthetic construct
  REGION 1..107: note = VL of TCB2-Cy06
DIVMTQSPSSLSASVGDRVTIRCITSCDIDDDMNWYQQKPGKAPKLLISEGNTLRPGVPSRFSGSGYGTDFTFTISSLQPEDIADYYCLQSDNLPYTFGGGTKLEIK

SEQ ID NO: 191 - protein, 107 aa, synthetic construct
  REGION 1..107: note = VL of TCB2-Cy07
DIVMTQSPSSLSASVGDRVTIRCITSTDIDDDMNWYQQKPGKAPKLLISEGNTLRPGVPSRFSGSGYGTDFTFTISSLQPEDIADYYCLQSCNLPYTFGGGTKLEIK

SEQ ID NO: 192 - protein, 107 aa, synthetic construct
  REGION 1..107: note = VL of TCB2-Cy08 to TCB2-Cy10
DIVMTQSPSSLSASVGDRVTIRCITSTDIDDDMNWYQQKPGKAPKLLISEGNTLRPGVPSRFSGSGYGTDFTFTISSLQPEDIADYYCLQSDCLPYTFGGGTKLEIK

SEQ ID NO: 193 - protein, 107 aa, synthetic construct
  REGION 1..107: note = VL of TCB2-Cy11
DIVMTQSPSSLSASVGDRVTIRCITSTDIDDDMNWYQQKPGKAPKLLISEGNTLRPGVPSRFSGSGYGTDFTFTISSLQPEDIADYYCLQSDNCPYTFGGGTKLEIK

SEQ ID NO: 194 - protein, 133 aa, synthetic construct
  REGION 1..133: note = The wild-type hIL-2 introduced with Cys substitution T111C
APTSSSTKKTQLQLEHLLLDLQMILNGINNYKNPKLTRMLTFKFYMPKKATELKHLQCLEEELKPLEEVLNLAQSKNFHLRPRDLISNINVIVLELKGSETTFMCEYADECATIVEFLNRWITFCQSIISTLT

SEQ ID NO: 195 - protein, 133 aa, synthetic construct
  REGION 1..133: note = The wild-type hIL-2 introduced with Cys substitution A73C
APTSSSTKKTQLQLEHLLLDLQMILNGINNYKNPKLTRMLTFKFYMPKKATELKHLQCLEEELKPLEEVLNLCQSKNFHLRPRDLISNINVIVLELKGSETTFMCEYADETATIVEFLNRWITFCQSIISTLT

SEQ ID NO: 196 - protein, 133 aa, synthetic construct
  REGION 1..133: note = The wild-type hIL-2 introduced with Cys substitution P34C
APTSSSTKKTQLQLEHLLLDLQMILNGINNYKNCKLTRMLTFKFYMPKKATELKHLQCLEEELKPLEEVLNLAQSKNFHLRPRDLISNINVIVLELKGSETTFMCEYADETATIVEFLNRWITFCQSIISTLT

SEQ ID NO: 197 - protein, 133 aa, synthetic construct
  REGION 1..133: note = The wild-type hIL-2 introduced with Cys substitution S75C
APTSSSTKKTQLQLEHLLLDLQMILNGINNYKNPKLTRMLTFKFYMPKKATELKHLQCLEEELKPLEEVLNLAQCKNFHLRPRDLISNINVIVLELKGSETTFMCEYADETATIVEFLNRWITFCQSIISTLT

SEQ ID NO: 198 - protein, 133 aa, synthetic construct
  REGION 1..133: note = The wild-type hIL-2 introduced with Cys substitution N77C
APTSSSTKKTQLQLEHLLLDLQMILNGINNYKNPKLTRMLTFKFYMPKKATELKHLQCLEEELKPLEEVLNLAQSKCFHLRPRDLISNINVIVLELKGSETTFMCEYADETATIVEFLNRWITFCQSIISTLT

SEQ ID NO: 199 - protein, 133 aa, synthetic construct
  REGION 1..133: note = The wild-type hIL-2 introduced with Cys substitution T37C
APTSSSTKKTQLQLEHLLLDLQMILNGINNYKNPKLCRMLTFKFYMPKKATELKHLQCLEEELKPLEEVLNLAQSKNFHLRPRDLISNINVIVLELKGSETTFMCEYADETATIVEFLNRWITFCQSIISTLT

SEQ ID NO: 200 - protein, 133 aa, synthetic construct
  REGION 1..133: note = The wild-type hIL-2 introduced with Cys substitution E68C
APTSSSTKKTQLQLEHLLLDLQMILNGINNYKNPKLTRMLTFKFYMPKKATELKHLQCLEEELKPLECVLNLAQSKNFHLRPRDLISNINVIVLELKGSETTFMCEYADETATIVEFLNRWITFCQSIISTLT

SEQ ID NO: 201 - protein, 133 aa, synthetic construct
  REGION 1..133: note = The wild-type hIL-2 introduced with Cys substitution T41C
APTSSSTKKTQLQLEHLLLDLQMILNGINNYKNPKLTRMLCFKFYMPKKATELKHLQCLEEELKPLEEVLNLAQSKNFHLRPRDLISNINVIVLELKGSETTFMCEYADETATIVEFLNRWITFCQSIISTLT

SEQ ID NO: 202 - protein, 133 aa, synthetic construct
  REGION 1..133: note = The wild-type hIL-2 introduced with Cys substitution F42C
APTSSSTKKTQLQLEHLLLDLQMILNGINNYKNPKLTRMLTCKFYMPKKATELKHLQCLEEELKPLEEVLNLAQSKNFHLRPRDLISNINVIVLELKGSETTFMCEYADETATIVEFLNRWITFCQSIISTLT

SEQ ID NO: 203 - protein, 133 aa, synthetic construct
  REGION 1..133: note = The wild-type hIL-2 introduced with Cys substitution R38C
APTSSSTKKTQLQLEHLLLDLQMILNGINNYKNPKLTCMLTFKFYMPKKATELKHLQCLEEELKPLEEVLNLAQSKNFHLRPRDLISNINVIVLELKGSETTFMCEYADETATIVEFLNRWITFCQSIISTLT

SEQ ID NO: 204 - protein, 133 aa, synthetic construct
  REGION 1..133: note = The wild-type hIL-2 introduced with Cys substitution D109C
APTSSSTKKTQLQLEHLLLDLQMILNGINNYKNPKLTRMLTFKFYMPKKATELKHLQCLEEELKPLEEVLNLAQSKNFHLRPRDLISNINVIVLELKGSETTFMCEYACETATIVEFLNRWITFCQSIISTLT

SEQ ID NO: 205 - protein, 133 aa, synthetic construct
  REGION 1..133: note = The wild-type hIL-2 introduced with Cys substitution L36C
APTSSSTKKTQLQLEHLLLDLQMILNGINNYKNPKCTRMLTFKFYMPKKATELKHLQCLEEELKPLEEVLNLAQSKNFHLRPRDLISNINVIVLELKGSETTFMCEYADETATIVEFLNRWITFCQSIISTLT

SEQ ID NO: 206 - protein, 264 aa, synthetic construct
  REGION 1..264: note = The first polypeptide of NARA1-Cy01
APTSSSTKKTQLQLEHLLLDLQMILNGINNYKNPKLTRMLTFKFYMPKKATELKHLQCLEEELKPLEEVLNLAQSKNFHLRPRDLISNINVIVLELKGSETTFMCEYADECATIVEFLNRWITFCQSIISTLTGGGGSGGGGSGGGGSGGGGSDIVLTQSPASLAVSLGQRATISCKASQSVDYDGDSYMNWYQQKPGQPPKLLIYAASNLESGIPARFSGSGSGTDFTLNIHPVEEEDAATYYCQQSNEDPYTFGGGTKLEIK

SEQ ID NO: 207 - protein, 264 aa, synthetic construct
  REGION 1..264: note = The first polypeptide of NARA1-Cy02
APTSSSTKKTQLQLEHLLLDLQMILNGINNYKNPKLTRMLTFKFYMPKKATELKHLQCLEEELKPLEEVLNLCQSKNFHLRPRDLISNINVIVLELKGSETTFMCEYADETATIVEFLNRWITFCQSIISTLTGGGGSGGGGSGGGGSGGGGSDIVLTQSPASLAVSLGQRATISCKASQSVDYDGDSYMNWYQQKPGQPPKLLIYAASNLESGIPARFSGSGSGTDFTLNIHPVEEEDAATYYCQQSNEDPYTFGGGTKLEIK

SEQ ID NO: 208 - protein, 264 aa, synthetic construct
  REGION 1..264: note = The first polypeptide of NARA1-Cy03
APTSSSTKKTQLQLEHLLLDLQMILNGINNYKNCKLTRMLTFKFYMPKKATELKHLQCLEEELKPLEEVLNLAQSKNFHLRPRDLISNINVIVLELKGSETTFMCEYADETATIVEFLNRWITFCQSIISTLTGGGGSGGGGSGGGGSGGGGSDIVLTQSPASLAVSLGQRATISCKASQSVDYDGDSYMNWYQQKPGQPPKLLIYAASNLESGIPARFSGSGSGTDFTLNIHPVEEEDAATYYCQQSNEDPYTFGGGTKLEIK

SEQ ID NO: 209 - protein, 264 aa, synthetic construct
  REGION 1..264: note = The first polypeptide of NARA1-Cy04
APTSSSTKKTQLQLEHLLLDLQMILNGINNYKNPKLTRMLTFKFYMPKKATELKHLQCLEEELKPLEEVLNLAQCKNFHLRPRDLISNINVIVLELKGSETTFMCEYADETATIVEFLNRWITFCQSIISTLTGGGGSGGGGSGGGGSGGGGSDIVLTQSPASLAVSLGQRATISCKASQSVDYCGDSYMNWYQQKPGQPPKLLIYAASNLESGIPARFSGSGSGTDFTLNIHPVEEEDAATYYCQQSNEDPYTFGGGTKLEIK

SEQ ID NO: 210 - protein, 264 aa, synthetic construct
  REGION 1..264: note = The first polypeptide of NARA1-Cy05
APTSSSTKKTQLQLEHLLLDLQMILNGINNYKNPKLTRMLTFKFYMPKKATELKHLQCLEEELKPLEEVLNLAQSKCFHLRPRDLISNINVIVLELKGSETTFMCEYADETATIVEFLNRWITFCQSIISTLTGGGGSGGGGSGGGGSGGGGSDIVLTQSPASLAVSLGQRATISCKASQSVDYCGDSYMNWYQQKPGQPPKLLIYAASNLESGIPARFSGSGSGTDFTLNIHPVEEEDAATYYCQQSNEDPYTFGGGTKLEIK

SEQ ID NO: 211 - protein, 264 aa, synthetic construct
  REGION 1..264: note = The first polypeptide of NARA1-Cy06
APTSSSTKKTQLQLEHLLLDLQMILNGINNYKNCKLTRMLTFKFYMPKKATELKHLQCLEEELKPLEEVLNLAQSKNFHLRPRDLISNINVIVLELKGSETTFMCEYADETATIVEFLNRWITFCQSIISTLTGGGGSGGGGSGGGGSGGGGSDIVLTQSPASLAVSLGQRATISCKASQSVDYDGDSYMNWYQQKPGQPPKLLIYAASNLESGIPARFSGSGSGTDFTLNIHPVEEEDAATYYCQQCNEDPYTFGGGTKLEIK

SEQ ID NO: 212 - protein, 264 aa, synthetic construct
  REGION 1..264: note = The first polypeptide of NARA1-Cy07
APTSSSTKKTQLQLEHLLLDLQMILNGINNYKNCKLTRMLTFKFYMPKKATELKHLQCLEEELKPLEEVLNLAQSKNFHLRPRDLISNINVIVLELKGSETTFMCEYADETATIVEFLNRWITFCQSIISTLTGGGGSGGGGSGGGGSGGGGSDIVLTQSPASLAVSLGQRATISCKASQSVDYDGDSYMNWYQQKPGQPPKLLIYAASNLESGIPARFSGSGSGTDFTLNIHPVEEEDAATYYCQQSCEDPYTFGGGTKLEIK

SEQ ID NO: 213 - protein, 264 aa, synthetic construct
  REGION 1..264: note = The first polypeptide of NARA1-Cy08
APTSSSTKKTQLQLEHLLLDLQMILNGINNYKNPKLCRMLTFKFYMPKKATELKHLQCLEEELKPLEEVLNLAQSKNFHLRPRDLISNINVIVLELKGSETTFMCEYADETATIVEFLNRWITFCQSIISTLTGGGGSGGGGSGGGGSGGGGSDIVLTQSPASLAVSLGQRATISCKASQSVDYDGDSYMNWYQQKPGQPPKLLIYAASNLESGIPARFSGSGSGTDFTLNIHPVEEEDAATYYCQQSNECPYTFGGGTKLEIK

SEQ ID NO: 214 - protein, 264 aa, synthetic construct
  REGION 1..264: note = The first polypeptide of NARA1-Cy09
APTSSSTKKTQLQLEHLLLDLQMILNGINNYKNPKLTRMLTFKFYMPKKATELKHLQCLEEELKPLECVLNLAQSKNFHLRPRDLISNINVIVLELKGSETTFMCEYADETATIVEFLNRWITFCQSIISTLTGGGGSGGGGSGGGGSGGGGSDIVLTQSPASLAVSLGQRATISCKASQSVDYDGDSYMNWYQQKPGQPPKLLIYAASNLESGIPARFSGSGSGTDFTLNIHPVEEEDAATYYCQQSNEDPYTFGGGTKLEIK

SEQ ID NO: 215 - protein, 264 aa, synthetic construct
  REGION 1..264: note = The first polypeptide of NARA1-Cy10
APTSSSTKKTQLQLEHLLLDLQMILNGINNYKNPKLTRMLCFKFYMPKKATELKHLQCLEEELKPLEEVLNLAQSKNFHLRPRDLISNINVIVLELKGSETTFMCEYADETATIVEFLNRWITFCQSIISTLTGGGGSGGGGSGGGGSGGGGSDIVLTQSPASLAVSLGQRATISCKASQSVDYDGDSYMNWYQQKPGQPPKLLIYAASNLESGIPARFSGSGSGTDFTLNIHPVEEEDAATYYCQQSNEDPYTFGGGTKLEIK

SEQ ID NO: 216 - protein, 264 aa, synthetic construct
  REGION 1..264: note = The first polypeptide of NARA1-Cy11
APTSSSTKKTQLQLEHLLLDLQMILNGINNYKNPKLTRMLTCKFYMPKKATELKHLQCLEEELKPLEEVLNLAQSKNFHLRPRDLISNINVIVLELKGSETTFMCEYADETATIVEFLNRWITFCQSIISTLTGGGGSGGGGSGGGGSGGGGSDIVLTQSPASLAVSLGQRATISCKASQSVDYDGDSYMNWYQQKPGQPPKLLIYAASNLESGIPARFSGSGSGTDFTLNIHPVEEEDAATYYCQQSNEDPYTFGGGTKLEIK

SEQ ID NO: 217 - protein, 260 aa, synthetic construct
  REGION 1..260: note = The first polypeptide of TCB2-Cy01 and TCB2-Cy03
APTSSSTKKTQLQLEHLLLDLQMILNGINNYKNPKLTRMLTFKFYMPKKATELKHLQCLEEELKPLECVLNLAQSKNFHLRPRDLISNINVIVLELKGSETTFMCEYADETATIVEFLNRWITFCQSIISTLTGGGGSGGGGSGGGGSGGGGSDIVMTQSPSSLSASVGDRVTIRCITSTDIDDDMNWYQQKPGKAPKLLISEGNTLRPGVPSRFSGSGYGTDFTFTISSLQPEDIADYYCLQSDNLPYTFGGGTKLEIK

SEQ ID NO: 218 - protein, 260 aa, synthetic construct
  REGION 1..260: note = The first polypeptide of TCB2-Cy02
APTSSSTKKTQLQLEHLLLDLQMILNGINNYKNPKLTRMLTCKFYMPKKATELKHLQCLEEELKPLEEVLNLAQSKNFHLRPRDLISNINVIVLELKGSETTFMCEYADETATIVEFLNRWITFCQSIISTLTGGGGSGGGGSGGGGSGGGGSDIVMTQSPSSLSASVGDRVTIRCITSTDIDDDMNWYQQKPGKAPKLLISEGNTLRPGVPSRFSGSGYGTDFTFTISSLQPEDIADYYCLQSDNLPYTFGGGTKLEIK

SEQ ID NO: 219 - protein, 260 aa, synthetic construct
  REGION 1..260: note = The first polypeptide of TCB2-Cy04
APTSSSTKKTQLQLEHLLLDLQMILNGINNYKNPKLTCMLTFKFYMPKKATELKHLQCLEEELKPLEEVLNLAQSKNFHLRPRDLISNINVIVLELKGSETTFMCEYADETATIVEFLNRWITFCQSIISTLTGGGGSGGGGSGGGGSGGGGSDIVMTQSPSSLSASVGDRVTIRCITSTDIDDDMNWYQQKPGKAPKLLISEGNTLRPGVPSRFSGSGYGTDFTFTISSLQPEDIADYYCLQSDNLPYTFGGGTKLEIK

SEQ ID NO: 220 - protein, 260 aa, synthetic construct
  REGION 1..260: note = The first polypeptide of TCB2-Cy05
APTSSSTKKTQLQLEHLLLDLQMILNGINNYKNPKLTRMLTFKFYMPKKATELKHLQCLEEELKPLEEVLNLAQSKNFHLRPRDLISNINVIVLELKGSETTFMCEYACETATIVEFLNRWITFCQSIISTLTGGGGSGGGGSGGGGSGGGGSDIVMTQSPSSLSASVGDRVTIRCITSTDIDDDMNWYQQKPGKAPKLLISEGNTLRPGVPSRFSGSGYGTDFTFTISSLQPEDIADYYCLQSDNLPYTFGGGTKLEIK

SEQ ID NO: 221 - protein, 260 aa, synthetic construct
  REGION 1..260: note = The first polypeptide of TCB2-Cy06
APTSSSTKKTQLQLEHLLLDLQMILNGINNYKNCKLTRMLTFKFYMPKKATELKHLQCLEEELKPLEEVLNLAQSKNFHLRPRDLISNINVIVLELKGSETTFMCEYADETATIVEFLNRWITFCQSIISTLTGGGGSGGGGSGGGGSGGGGSDIVMTQSPSSLSASVGDRVTIRCITSCDIDDDMNWYQQKPGKAPKLLISEGNTLRPGVPSRFSGSGYGTDFTFTISSLQPEDIADYYCLQSDNLPYTFGGGTKLEIK

SEQ ID NO: 222 - protein, 260 aa, synthetic construct
  REGION 1..260: note = The first polypeptide of TCB2-Cy07
APTSSSTKKTQLQLEHLLLDLQMILNGINNYKNCKLTRMLTFKFYMPKKATELKHLQCLEEELKPLEEVLNLAQSKNFHLRPRDLISNINVIVLELKGSETTFMCEYADETATIVEFLNRWITFCQSIISTLTGGGGSGGGGSGGGGSGGGGSDIVMTQSPSSLSASVGDRVTIRCITSTDIDDDMNWYQQKPGKAPKLLISEGNTLRPGVPSRFSGSGYGTDFTFTISSLQPEDIADYYCLQSCNLPYTFGGGTKLEIK

SEQ ID NO: 223 - protein, 260 aa, synthetic construct
  REGION 1..260: note = The first polypeptide of TCB2-Cy08
APTSSSTKKTQLQLEHLLLDLQMILNGINNYKNCKLTRMLTFKFYMPKKATELKHLQCLEEELKPLEEVLNLAQSKNFHLRPRDLISNINVIVLELKGSETTFMCEYADETATIVEFLNRWITFCQSIISTLTGGGGSGGGGSGGGGSGGGGSDIVMTQSPSSLSASVGDRVTIRCITSTDIDDDMNWYQQKPGKAPKLLISEGNTLRPGVPSRFSGSGYGTDFTFTISSLQPEDIADYYCLQSDCLPYTFGGGTKLEIK

SEQ ID NO: 224 - protein, 260 aa, synthetic construct
  REGION 1..260: note = The first polypeptide of TCB2-Cy09
APTSSSTKKTQLQLEHLLLDLQMILNGINNYKNPKCTRMLTFKFYMPKKATELKHLQCLEEELKPLEEVLNLAQSKNFHLRPRDLISNINVIVLELKGSETTFMCEYADETATIVEFLNRWITFCQSIISTLTGGGGSGGGGSGGGGSGGGGSDIVMTQSPSSLSASVGDRVTIRCITSTDIDDDMNWYQQKPGKAPKLLISEGNTLRPGVPSRFSGSGYGTDFTFTISSLQPEDIADYYCLQSDCLPYTFGGGTKLEIK

SEQ ID NO: 225 - protein, 260 aa, synthetic construct
  REGION 1..260: note = The first polypeptide of TCB2-Cy10
APTSSSTKKTQLQLEHLLLDLQMILNGINNYKNPKLCRMLTFKFYMPKKATELKHLQCLEEELKPLEEVLNLAQSKNFHLRPRDLISNINVIVLELKGSETTFMCEYADETATIVEFLNRWITFCQSIISTLTGGGGSGGGGSGGGGSGGGGSDIVMTQSPSSLSASVGDRVTIRCITSTDIDDDMNWYQQKPGKAPKLLISEGNTLRPGVPSRFSGSGYGTDFTFTISSLQPEDIADYYCLQSDCLPYTFGGGTKLEIK

SEQ ID NO: 226 - protein, 260 aa, synthetic construct
  REGION 1..260: note = The first polypeptide of TCB2-Cy11
APTSSSTKKTQLQLEHLLLDLQMILNGINNYKNPKLCRMLTFKFYMPKKATELKHLQCLEEELKPLEEVLNLAQSKNFHLRPRDLISNINVIVLELKGSETTFMCEYADETATIVEFLNRWITFCQSIISTLTGGGGSGGGGSGGGGSGGGGSDIVMTQSPSSLSASVGDRVTIRCITSTDIDDDMNWYQQKPGKAPKLLISEGNTLRPGVPSRFSGSGYGTDFTFTISSLQPEDIADYYCLQSDNCPYTFGGGTKLEIK

SEQ ID NO: 227 - protein, 330 aa, synthetic construct
  REGION 1..330: note = The wild-type IgG1 constant region
ASTKGPSVFPLAPSSKSTSGGTAALGCLVKDYFPEPVTVSWNSGALTSGVHTFPAVLQSSGLYSLSSVVTVPSSSLGTQTYICNVNHKPSNTKVDKRVEPKSCDKTHTCPPCPAPELLGGPSVFLFPPKPKDTLMISRTPEVTCVVVDVSHEDPEVKFNWYVDGVEVHNAKTKPREEQYNSTYRVVSVLTVLHQDWLNGKEYKCKVSNKALPAPIEKTISKAKGQPREPQVYTLPPSRDELTKNQVSLTCLVKGFYPSDIAVEWESNGQPENNYKTTPPVLDSDGSFFLYSKLTVDKSRWQQGNVFSCSVMHEALHNHYTQKSLSLSPGK

SEQ ID NO: 228 - protein, 330 aa, synthetic construct
  REGION 1..330: note = IgG1 constant region / pI TM mutant
ASTKGPSVFPLAPSSKSTSGGTAALGCLVKDYFPEPVTVSWNSGALTSGVHTFPAVLQSSGLYSLSSVVTVPSSSLGTQTYICNVDHKPSNTKVDKRVEPKSCDKTHTCPPCPAPEFEGGPSVFLFPPKPKDTLMISRTPEVTCVVVDVSHEDPEVQFNWYVDGVEVHNAKTKPREEQYNSTYRVVSVLTVLHQDWLNGKEYKCKVSNKALPASIEKTISKAKGQPREPQVYTLPPSRDELTKNQVSLTCLVKGFYPSDIAVEWESNGQPENNYKTTPPVLDSDGSFFLYSKLTVDKSRWQEGNVFSCSVMHEALHNHYTQKSLSLSPGK

SEQ ID NO: 229 - protein, 153 aa, synthetic construct
  REGION 1..153: note = Full-length human IL-2 (comprising signal peptide)
MYRMQLLSCIALSLALVTNSAPTSSSTKKTQLQLEHLLLDLQMILNGINNYKNPKLTRMLTFKFYMPKKATELKHLQCLEEELKPLEEVLNLAQSKNFHLRPRDLISNINVIVLELKGSETTFMCEYADETATIVEFLNRWITFCQSIISTLT

SEQ ID NO: 230 - protein, 17 aa, synthetic construct
  REGION 1..17: note = HCDR2
  MUTAGEN 5: note = Z at position 5 is Z1 and represents E or D
  MUTAGEN 17: note = X at position 17 is X3 and represents N, S or G
RIDPZDDSTKYAENFKX

SEQ ID NO: 231 - protein, 14 aa, synthetic construct
  REGION 1..14: note = HCDR3
  MUTAGEN 1: note = Z at position 1 is Z2 and represents V, I, R or T
  MUTAGEN 4: note = Z at positin 4 is Z3 and represents Y, L, H or W
  MUTAGEN 6: note = Z at position 6 is Z4 and represents S, T, A, R, N, D, Q, E, H, I, L, K, F, P, W, Y or V
ZTFZYZRELRWFAY

SEQ ID NO: 232 - protein, 11 aa, synthetic construct
  REGION 1..11: note = LCDR1
  MUTAGEN 5: note = Z at position 5 is Z5 and represents D, Y, N, H, I, L or F
  MUTAGEN 7: note = Z at position 7 is Z6 and represents G, S, A, R, N, Q, I, L, T or D
QASQZIZNYLS

SEQ ID NO: 233 - protein, 7 aa, synthetic construct
  REGION 1..7: note = LCDR2
  MUTAGEN 1: note = Z at position 1 is Z7 and represents S, Q, R, T, W or Y
  MUTAGEN 3: note = Z at position 3 is Z8 and represents T or G
  MUTAGEN 7: note = X at position 7 is X4 and represnts D, S or T
ZAZSLAX

SEQ ID NO: 234 - protein, 14 aa, synthetic construct
  REGION 1..14: note = HCDR3
  MUTAGEN 1: note = Z at position 1 is Z2 and represents V or I
  MUTAGEN 3: note = X at position 3 is XII and represents F or C
  MUTAGEN 4: note = Z at position 4 is Z3 and represents Y or L
  MUTAGEN 6: note = Z at position 6 is Z4 and represnts S or T
ZTXZYZRELRWFAY

SEQ ID NO: 235 - protein, 11 aa, synthetic construct
  REGION 1..11: note = LCDR1
  MUTAGEN 5: note = Z at position 5 is Z5 and represents D or Y
  MUTAGEN 7: note = Z at position 7 is Z6 and represents G, S or C
  MUTAGEN 8: note = X at position 8 is XI and represents N or C
  MUTAGEN 9: note = X at position 9 is XIV and represents Y or C
QASQZIZXXLS

SEQ ID NO: 236 - protein, 7 aa, synthetic construct
  REGION 1..7: note = LCDR2
  MUTAGEN 1: note = Z at position 1 is Z7 and represnts S, Q or C
  MUTAGEN 3: note = Z at position 3 is Z8 and represents T or C
  MUTAGEN 7: note = X at position 7 is X4 and represents S
ZAZSLAX

SEQ ID NO: 237 - protein, 9 aa, synthetic construct
  REGION 1..9: note = LCDR3
  MUTAGEN 4: note = X at position 4 is XIII and represnts Y or C
LQHXSTPYT